European Patent Specification EP 3 911 348 B1, published January 28, 2026. Title: METHOD OF TREATING CENTRAL NERVOUS SYSTEM DISEASE. Applicant: L & J Bio Co., Ltd. The sequence listing filed with the application follows.

SEQUENCE LISTING (7 sequences)

SEQ ID NO: 1 - protein, 5 aa, Artificial Sequence
  GS linker
GGSAS

SEQ ID NO: 2 - protein, 8 aa, Artificial Sequence
  GS linker
GGGSGGGS

SEQ ID NO: 3 - protein, 4 aa, Artificial Sequence
  cleavable linker
GFLG

SEQ ID NO: 4 - protein, 10 aa, Artificial Sequence
  cleavable linker
GFLGGGGSAS

SEQ ID NO: 5 - DNA, 2211 bp, Artificial Sequence
  AL04
tccagccctggcaagccccctcgcctggtgggcggccccatggacgccagcgtggaggaggagggcgtgaggcgggctctggacttcgccgtgggcgagtacaacaaggcctccaatgatatgtatcactctagggctctgcaggtggtgagagcccgcaagcagatcgtggctggcgtgaactacttcctggatgtggagctgggcaggaccacatgcaccaagacacagccaaacctggacaattgtccttttcacgatcagccacatctgaagcggaaggccttctgctcttttcagatctatgctgtgccctggcagggcaccatgacactgtctaagtccacctgtcaggacgctggcggctccgctagcgatgctcacaagtctgaggtggcccataggttcaaggacctgggcgaggagaactttaaggccctggtgctgatcgctttcgcccagtacctgcagcagtgcccttttgaggaccacgtgaagctggtgaacgaggtgaccgagttcgctaagacatgcgtggctgacgagagcgccgagaattgtgataagtctctgcataccctgtttggcgataagctgtgcaccgtggccacactgagagagacatatggcgagatggctgactgctgtgccaagcaggagccagagcgcaacgagtgcttcctgcagcacaaggacgataaccccaatctgcctagactggtgcgcccagaggtggacgtgatgtgcaccgctttccacgataatgaggagacatttctgaagaagtacctgtatgagatcgccaggcggcatccttacttttatgctccagagctgctgttctttgccaagagatacaaggccgctttcaccgagtgctgtcaggccgctgataaggccgcttgcctgctgcccaagctggacgagctgagagatgagggcaaggcttccagcgccaagcagcgcctgaagtgtgcttccctgcagaagttcggcgagagagcctttaaggcttgggctgtggctaggctgagccagcggttccctaaggctgagtttgccgaggtgtctaagctggtgaccgacctgacaaaggtgcacaccgagtgctgtcatggcgacctgctggagtgcgccgacgatagggctgatctggccaagtacatctgtgagaaccaggactctatctcttccaagctgaaggagtgctgtgagaagccactgctggagaagtcccattgcatcgctgaggtggagaacgacgagatgccagctgatctgccctccctggccgctgactttgtggagagcaaggacgtgtgcaagaattacgccgaggctaaggacgtgttcctgggcatgtttctgtacgagtatgctagacgccaccctgactacagcgtggtgctgctgctgagactggccaagacctatgagaccacactggagaagtgctgtgccgctgccgatccacatgagtgctatgctaaggtgttcgacgagtttaagcccctggtggaggagcctcagaacctgatcaagcagaattgtgagctgtttgagcagctgggcgagtacaagttccagaacgccctgctggtgcgctatacaaagaaggtgccacaggtgtctacccccacactggtggaggtgtccaggaatctgggcaaggtcggcagcaagtgctgtaagcaccctgaggctaagcggatgccatgcgccgaggattacctgtccgtggtgctgaatcagctgtgcgtgctgcatgagaagaccccagtgagcgacagggtgaccaagtgctgtacagagtctctggtgaacaggcggccctgcttttccgctctggaggtggatgagacatatgtgcctaaggagttcaatgctgagaccttcacatttcacgccgacatctgtaccctgagcgagaaggagcggcagatcaagaagcagacagccctggtggagctggtgaagcataagcccaaggctaccaaggagcagctgaaggccgtgatggacgatttcgctgcctttgtggagaagtgctgtaaggctgacgataaggagacatgctttgccgaggagggcaagaagctggtggctgcctctcaggctgccctgggactgggcttcctgggatacgctaggaaggctgctaggcaggcccgggcttatgctaggaaggctgctagacaggctcgcgccggc

SEQ ID NO: 6 - protein, 737 aa, Artificial Sequence
  AL04
SSPGKPPRLVGGPMDASVEEEGVRRALDFAVGEYNKASNDMYHSRALQVVRARKQIVAGVNYFLDVELGRTTCTKTQPNLDNCPFHDQPHLKRKAFCSFQIYAVPWQGTMTLSKSTCQDAGGSASDAHKSEVAHRFKDLGEENFKALVLIAFAQYLQQCPFEDHVKLVNEVTEFAKTCVADESAENCDKSLHTLFGDKLCTVATLRETYGEMADCCAKQEPERNECFLQHKDDNPNLPRLVRPEVDVMCTAFHDNEETFLKKYLYEIARRHPYFYAPELLFFAKRYKAAFTECCQAADKAACLLPKLDELRDEGKASSAKQRLKCASLQKFGERAFKAWAVARLSQRFPKAEFAEVSKLVTDLTKVHTECCHGDLLECADDRADLAKYICENQDSISSKLKECCEKPLLEKSHCIAEVENDEMPADLPSLAADFVESKDVCKNYAEAKDVFLGMFLYEYARRHPDYSVVLLLRLAKTYETTLEKCCAAADPHECYAKVFDEFKPLVEEPQNLIKQNCELFEQLGEYKFQNALLVRYTKKVPQVSTPTLVEVSRNLGKVGSKCCKHPEAKRMPCAEDYLSVVLNQLCVLHEKTPVSDRVTKCCTESLVNRRPCFSALEVDETYVPKEFNAETFTFHADICTLSEKERQIKKQTALVELVKHKPKATKEQLKAVMDDFAAFVEKCCKADDKETCFAEEGKKLVAASQAALGLGFLGYARKAARQARAYARKAARQARAG

SEQ ID NO: 7 - protein, 441 aa, Homo sapiens
MAEPRQEFEVMEDHAGTYGLGDRKDQGGYTMHQDQEGDTDAGLKESPLQTPTEDGSEEPGSETSDAKSTPTAEDVTAPLVDEGAPGKQAAAQPHTEIPEGTTAEEAGIGDTPSLEDEAAGHVTQARMVSKSKDGTGSDDKKAKGADGKTKIATPRGAAPPGQKGQANATRIPAKTPPAPKTPPSSGEPPKSGDRSGYSSPGSPGTPGSRSRTPSLPTPPTREPKKVAVVRTPPKSPSSAKSRLQTAPVPMPDLKNVKSKIGSTENLKHQPGGGKVQIINKKLDLSNVQSKCGSKDNIKHVPGGGSVQIVYKPVDLSKVTSKCGSLGNIHHKPGGGQVEVKSEKLDFKDRVQSKIGSLDNITHVPGGGNKKIETHKLTFRENAKAKTDHGAEIVYKSPVVSGDTSPRHLSNVSSTGSIDMVDSPQLATLADEVSASLAKQGL